European Patent Application EP 4 467 646 A1, published November 27, 2024. Title: Cell Sheet. Applicant: OSAKA UNIVERSITY. The sequence listing filed with the application follows.

SEQUENCE LISTING (6 sequences)

SEQ ID NO: 1 - DNA, 8835 bp, Homo sapiens
  source 1..8835: mol_type = genomic DNA
atgacgctgcggcttctggtggccgcgctctgcgccgggatcctggcagaggcgccccgagtgcgagcccagcacagggagagagtgacctgcacgcgcctttacgccgctgacattgtgttcttactggatggctcctcatccattggccgcagcaatttccgcgaggtccgcagctttctcgaagggctggtgctgcctttctctggagcagccagtgcacagggtgtgcgctttgccacagtgcagtacagcgatgatccacggacagagttcggcctggatgcacttggctctgggggtgatgtgatccgcgccatccgtgagcttagctacaaggggggcaacactcgcacaggggctgcaattctccatgtggctgaccatgtcttcctgccccagctggcccgacctggtgtccccaaggtctgcatcctgatcacagacgggaagtcccaggacctggtggacacagctgcccaaaggctgaaggggcagggggtcaagctatttgctgtggggatcaagaatgctgaccctgaggagctgaagcgagttgcctcacagcccaccagtgacttcttcttcttcgtcaatgacttcagcatcttgaggacactactgcccctcgtttcccggagagtgtgcacgactgctggtggcgtgcctgtgacccgacctccggatgactcgacctctgctccacgagacctggtgctgtctgagccaagcagccaatccttgagagtacagtggacagcggccagtggccctgtgactggctacaaggtccagtacactcctctgacggggctgggacagccactgccgagtgagcggcaggaggtgaacgtcccagctggtgagaccagtgtgcggctgcggggtctccggccactgaccgagtaccaagtgactgtgattgccctctacgccaacagcatcggggaggctgtgagcgggacagctcggaccactgccctagaagggccggaactgaccatccagaataccacagcccacagcctcctggtggcctggcggagtgtgccaggtgccactggctaccgtgtgacatggcgggtcctcagtggtgggcccacacagcagcaggagctgggccctgggcagggttcagtgttgctgcgtgacttggagcctggcacggactatgaggtgaccgtgagcaccctatttggccgcagtgtggggcccgccacttccctgatggctcgcactgacgcttctgttgagcagaccctgcgcccggtcatcctgggccccacatccatcctcctttcctggaacttggtgcctgaggcccgtggctaccggttggaatggcggcgtgagactggcttggagccaccgcagaaggtggtactgccctctgatgtgacccgctaccagttggatgggctgcagccgggcactgagtaccgcctcacactctacactctgctggagggccacgaggtggccacccctgcaaccgtggttcccactggaccagagctgcctgtgagccctgtaacagacctgcaagccaccgagctgcccgggcagcgggtgcgagtgtcctggagcccagtccctggtgccacccagtaccgcatcattgtgcgcagcacccagggggttgagcggaccctggtgcttcctgggagtcagacagcattcgacttggatgacgttcaggctgggcttagctacactgtgcgggtgtctgctcgagtgggtccccgtgagggcagtgccagtgtcctcactgtccgccgggagccggaaactccacttgctgttccagggctgcgggttgtggtgtcagatgcaacgcgagtgagggtggcctggggacccgtccctggagccagtggatttcggattagctggagcacaggcagtggtccggagtccagccagacactgcccccagactctactgccacagacatcacagggctgcagcctggaaccacctaccaggtggctgtgtcggtactgcgaggcagagaggagggccctgctgcagtcatcgtggctcgaacggacccactgggcccagtgaggacggtccatgtgactcaggccagcagctcatctgtcaccattacctggaccagggttcctggcgccacaggatacagggtttcctggcactcagcccacggcccagagaaatcccagttggtttctggggaggccacggtggctgagctggatggactggagccagatactgagtatacggtgcatgtgagggcccatgtggctggcgtggatgggccccctgcctctgtggttgtgaggactgcccctgagcctgtgggtcgtgtgtcgaggctgcagatcctcaatgcttccagcgacgttctacggatcacctgggtaggggtcactggagccacagcttacagactggcctggggccggagtgaaggcggccccatgaggcaccagatactcccaggaaacacagactctgcagagatccggggtctcgaaggtggagtcagctactcagtgcgagtgactgcacttgtcggggaccgcgagggcacacctgtctccattgttgtcactacgccgcctgaggctccgccagccctggggacgcttcacgtggtgcagcgcggggagcactcgctgaggctgcgctgggagccggtgcccagagcgcagggcttccttctgcactggcaacctgagggtggccaggaacagtcccgggtcctggggcccgagctcagcagctatcacctggacgggctggagccagcgacacagtaccgcgtgaggctgagtgtcctagggccagctggagaagggccctctgcagaggtgactgcgcgcactgagtcacctcgtgttccaagcattgaactacgtgtggtggacacctcgatcgactcggtgactttggcctggactccagtgtccagggcatccagctacatcctatcctggcggccactcagaggccctggccaggaagtgcctgggtccccgcagacacttccagggatctcaagctcccagcgggtgacagggctagagcctggcgtctcttacatcttctccctgacgcctgtcctggatggtgtgcggggtcctgaggcatctgtcacacagacgccagtgtgcccccgtggcctggcggatgtggtgttcctaccacatgccactcaagacaatgctcaccgtgcggaggctacgaggagggtcctggagcgtctggtgttggcacttgggcctcttgggccacaggcagttcaggttggcctgctgtcttacagtcatcggccctccccactgttcccactgaatggctcccatgaccttggcattatcttgcaaaggatccgtgacatgccctacatggacccaagtgggaacaacctgggcacagccgtggtcacagctcacagatacatgttggcaccagatgctcctgggcgccgccagcacgtaccaggggtgatggttctgctagtggatgaacccttgagaggtgacatattcagccccatccgtgaggcccaggcttctgggcttaatgtggtgatgttgggaatggctggagcggacccagagcagctgcgtcgcttggcgccgggtatggactctgtccagaccttcttcgccgtggatgatgggccaagcctggaccaggcagtcagtggtctggccacagccctgtgtcaggcatccttcactactcagccccggccagagccctgcccagtgtattgtccaaagggccagaagggggaacctggagagatgggcctgagaggacaagttgggcctcctggcgaccctggcctcccgggcaggaccggtgctcccggcccccaggggccccctggaagtgccactgccaagggcgagaggggcttccctggagcagatgggcgtccaggcagccctggccgcgccgggaatcctgggacccctggagcccctggcctaaagggctctccagggttgcctggccctcgtggggacccgggagagcgaggacctcgaggcccaaagggggagccgggggctcccggacaagtcatcggaggtgaaggacctgggcttcctgggcggaaaggggaccctggaccatcgggcccccctggacctcgtggaccactgggggacccaggaccccgtggccccccagggcttcctggaacagccatgaagggtgacaaaggcgatcgtggggagcggggtccccctggaccaggtgaaggtggcattgctcctggggagcctgggctgccgggtcttcccggaagccctggaccccaaggccccgttggcccccctggaaagaaaggagaaaaaggtgactctgaggatggagctccaggcctcccaggacaacctgggtctccgggtgagcagggcccacggggacctcctggagctattggccccaaaggtgaccggggctttccagggcccctgggtgaggctggagagaagggcgaacgtggacccccaggcccagcgggatcccgggggctgccaggggttgctggacgtcctggagccaagggtcctgaagggccaccaggacccactggccgccaaggagagaagggggagcctggtcgccctggggaccctgcagtggtgggacctgctgttgctggacccaaaggagaaaagggagatgtggggcccgctgggcccagaggagctaccggagtccaaggggaacggggcccacccggcttggttcttcctggagaccctggccccaagggagaccctggagaccggggtcccattggccttactggcagagcaggacccccaggtgactcagggcctcctggagagaagggagaccctgggcggcctggccccccaggacctgttggcccccgaggacgagatggtgaagttggagagaaaggtgacgagggtcctccgggtgacccgggtttgcctggaaaagcaggcgagcgtggccttcggggggcacctggagttcgggggcctgtgggtgaaaagggagaccagggagatcctggagaggatggacgaaatggcagccctggatcatctggacccaagggtgaccgtggggagccgggtcccccaggacccccgggacggctggtagacacaggacctggagccagagagaagggagagcctggggaccgcggacaagagggtcctcgagggcccaagggtgatcctggcctccctggagcccctggggaaaggggcattgaagggtttcggggacccccaggcccacagggggacccaggtgtccgaggcccagcaggagaaaagggtgaccggggtccccctgggctggatggccggagcggactggatgggaaaccaggagccgctgggccctctgggccgaatggtgctgcaggcaaagctggggacccagggagagacgggcttccaggcctccgtggagaacagggcctccctggcccctctggtccccctggattaccgggaaagccaggcgaggatggcaaacctggcctgaatggaaaaaacggagaacctggggaccctggagaagacgggaggaagggagagaaaggagattcaggcgcctctgggagagaaggtcgtgatggccccaagggtgagcgtggagctcctggtatccttggaccccaggggcctccaggcctcccagggccagtgggccctcctggccagggttttcctggtgtcccaggaggcacgggccccaagggtgaccgtggggagactggatccaaaggggagcagggcctccctggagagcgtggcctgcgaggagagcctggaagtgtgccgaatgtggatcggttgctggaaactgctggcatcaaggcatctgccctgcgggagatcgtggagacctgggatgagagctctggtagcttcctgcctgtgcccgaacggcgtcgaggccccaagggggactcaggcgaacagggccccccaggcaaggagggccccatcggctttcctggagaacgcgggctgaagggcgaccgtggagaccctggccctcaggggccacctggtctggcccttggggagaggggcccccccgggccttccggccttgccggggagcctggaaagcctggtattcccgggctcccaggcagggctgggggtgtgggagaggcaggaaggccaggagagaggggagaacggggagagaaaggagaacgtggagaacagggcagagatggccctcctggactccctggaacccctgggccccccggaccccctggccccaaggtgtctgtggatgagccaggtcctggactctctggagaacagggaccccctggactcaagggtgctaagggggagccgggcagcaatggtgaccaaggtcccaaaggagacaggggtgtgccaggcatcaaaggagaccggggagagcctggaccgaggggtcaggacggcaacccgggtctaccaggagagcgtggtatggctgggcctgaagggaagccgggtctgcagggtccaagaggcccccctggcccagtgggtggtcatggagaccctggaccacctggtgccccgggtcttgctggccctgcaggaccccaaggaccttctggcctgaagggggagcctggagagacaggacctccaggacggggcctgactggacctactggagctgtgggacttcctggaccccccggcccttcaggccttgtgggtccacaggggtctccaggtttgcctggacaagtgggggagacagggaagccgggagccccaggtcgagatggtgccagtggaaaagatggagacagagggagccctggtgtgccagggtcaccaggtctgcctggccctgtcggacctaaaggagaacctggccccacgggggcccctggacaggctgtggtcgggctccctggagcaaagggagagaagggagcccctggaggccttgctggagacctggtgggtgagccgggagccaaaggtgaccgaggactgccagggccgcgaggcgagaagggtgaagctggccgtgcaggggagcccggagaccctggggaagatggtcagaaaggggctccaggacccaaaggtttcaagggtgacccaggagtcggggtcccgggctcccctgggcctcctggccctccaggtgtgaagggagatctgggcctccctggcctgcccggtgctcctggtgttgttgggttcccgggtcagacaggccctcgaggagagatgggtcagccaggccctagtggagagcggggtctggcaggccccccagggagagaaggaatcccaggacccctggggccacctggaccaccggggtcagtgggaccacctggggcctctggactcaaaggagacaagggagaccctggagtagggctgcctgggccccgaggcgagcgtggggagccaggcatccggggtgaagatggccgccccggccaggagggaccccgaggactcacggggccccctggcagcaggggagagcgtggggagaagggtgatgttgggagtgcaggactaaagggtgacaagggagactcagctgtgatcctggggcctccaggcccacggggtgccaagggggacatgggtgaacgagggcctcggggcttggatggtgacaaaggacctcggggagacaatggggaccctggtgacaagggcagcaagggagagcctggtgacaagggctcagccgggttgccaggactgcgtggactcctgggaccccagggtcaacctggtgcagcagggatccctggtgacccgggatccccaggaaaggatggagtgcctggtatccgaggagaaaaaggagatgttggcttcatgggtccccggggcctcaagggtgaacggggagtgaagggagcctgtggccttgatggagagaagggagacaagggagaagctggtcccccaggccgccccgggctggcaggacacaaaggagagatgggggagcctggtgtgccgggccagtcgggggcccctggcaaggagggcctgatcggtcccaagggtgaccgaggctttgacgggcagccaggccccaagggtgaccagggcgagaaaggggagcggggaaccccaggaattgggggcttcccaggccccagtggaaatgatggctctgctggtcccccagggccacctggcagtgttggtcccagaggccccgaaggacttcagggccagaagggtgagcgaggtccccccggagagagagtggtgggggctcctggggtccctggagctcctggcgagagaggggagcaggggcggccagggcctgccggtcctcgaggcgagaagggagaagctgcactgacggaggatgacatccggggctttgtgcgccaagagatgagtcagcactgtgcctgccagggccagttcatcgcatctggatcacgacccctccctagttatgctgcagacactgccggctcccagctccatgctgtgcctgtgctccgcgtctctcatgcagaggaggaagagcgggtaccccctgaggatgatgagtactctgaatactccgagtattctgtggaggagtaccaggaccctgaagctccttgggatagtgatgacccctgttccctgccactggatgagggctcctgcactgcctacaccctgcgctggtaccatcgggctgtgacaggcagcacagaggcctgtcacccttttgtctatggtggctgtggagggaatgccaaccgttttgggacccgtgaggcctgcgagcgccgctgcccaccccgggtggtccagagccaggggacaggtactgcccaggactga

SEQ ID NO: 2 - protein, 2944 aa, Homo sapiens
MTLRLLVAALCAGILAEAPRVRAQHRERVTCTRLYAADIVFLLDGSSSIGRSNFREVRSFLEGLVLPFSGAASAQGVRFATVQYSDDPRTEFGLDALGSGGDVIRAIRELSYKGGNTRTGAAILHVADHVFLPQLARPGVPKVCILITDGKSQDLVDTAAQRLKGQGVKLFAVGIKNADPEELKRVASQPTSDFFFFVNDFSILRTLLPLVSRRVCTTAGGVPVTRPPDDSTSAPRDLVLSEPSSQSLRVQWTAASGPVTGYKVQYTPLTGLGQPLPSERQEVNVPAGETSVRLRGLRPLTEYQVTVIALYANSIGEAVSGTARTTALEGPELTIQNTTAHSLLVAWRSVPGATGYRVTWRVLSGGPTQQQELGPGQGSVLLRDLEPGTDYEVTVSTLFGRSVGPATSLMARTDASVEQTLRPVILGPTSILLSWNLVPEARGYRLEWRRETGLEPPQKVVLPSDVTRYQLDGLQPGTEYRLTLYTLLEGHEVATPATVVPTGPELPVSPVTDLQATELPGQRVRVSWSPVPGATQYRIIVRSTQGVERTLVLPGSQTAFDLDDVQAGLSYTVRVSARVGPREGSASVLTVRREPETPLAVPGLRVVVSDATRVRVAWGPVPGASGFRISWSTGSGPESSQTLPPDSTATDITGLQPGTTYQVAVSVLRGREEGPAAVIVARTDPLGPVRTVHVTQASSSSVTITWTRVPGATGYRVSWHSAHGPEKSQLVSGEATVAELDGLEPDTEYTVHVRAHVAGVDGPPASVVVRTAPEPVGRVSRLQILNASSDVLRITWVGVTGATAYRLAWGRSEGGPMRHQILPGNTDSAEIRGLEGGVSYSVRVTALVGDREGTPVSIVVTTPPEAPPALGTLHVVQRGEHSLRLRWEPVPRAQGFLLHWQPEGGQEQSRVLGPELSSYHLDGLEPATQYRVRLSVLGPAGEGPSAEVTARTESPRVPSIELRVVDTSIDSVTLAWTPVSRASSYILSWRPLRGPGQEVPGSPQTLPGISSSQRVTGLEPGVSYIFSLTPVLDGVRGPEASVTQTPVCPRGLADVVFLPHATQDNAHRAEATRRVLERLVLALGPLGPQAVQVGLLSYSHRPSPLFPLNGSHDLGIILQRIRDMPYMDPSGNNLGTAVVTAHRYMLAPDAPGRRQHVPGVMVLLVDEPLRGDIFSPIREAQASGLNVVMLGMAGADPEQLRRLAPGMDSVQTFFAVDDGPSLDQAVSGLATALCQASFTTQPRPEPCPVYCPKGQKGEPGEMGLRGQVGPPGDPGLPGRTGAPGPQGPPGSATAKGERGFPGADGRPGSPGRAGNPGTPGAPGLKGSPGLPGPRGDPGERGPRGPKGEPGAPGQVIGGEGPGLPGRKGDPGPSGPPGPRGPLGDPGPRGPPGLPGTAMKGDKGDRGERGPPGPGEGGIAPGEPGLPGLPGSPGPQGPVGPPGKKGEKGDSEDGAPGLPGQPGSPGEQGPRGPPGAIGPKGDRGFPGPLGEAGEKGERGPPGPAGSRGLPGVAGRPGAKGPEGPPGPTGRQGEKGEPGRPGDPAVVGPAVAGPKGEKGDVGPAGPRGATGVQGERGPPGLVLPGDPGPKGDPGDRGPIGLTGRAGPPGDSGPPGEKGDPGRPGPPGPVGPRGRDGEVGEKGDEGPPGDPGLPGKAGERGLRGAPGVRGPVGEKGDQGDPGEDGRNGSPGSSGPKGDRGEPGPPGPPGRLVDTGPGAREKGEPGDRGQEGPRGPKGDPGLPGAPGERGIEGFRGPPGPQGDPGVRGPAGEKGDRGPPGLDGRSGLDGKPGAAGPSGPNGAAGKAGDPGRDGLPGLRGEQGLPGPSGPPGLPGKPGEDGKPGLNGKNGEPGDPGEDGRKGEKGDSGASGREGRDGPKGERGAPGILGPQGPPGLPGPVGPPGQGFPGVPGGTGPKGDRGETGSKGEQGLPGERGLRGEPGSVPNVDRLLETAGIKASALREIVETWDESSGSFLPVPERRRGPKGDSGEQGPPGKEGPIGFPGERGLKGDRGDPGPQGPPGLALGERGPPGPSGLAGEPGKPGIPGLPGRAGGVGEAGRPGERGERGEKGERGEQGRDGPPGLPGTPGPPGPPGPKVSVDEPGPGLSGEQGPPGLKGAKGEPGSNGDQGPKGDRGVPGIKGDRGEPGPRGQDGNPGLPGERGMAGPEGKPGLQGPRGPPGPVGGHGDPGPPGAPGLAGPAGPQGPSGLKGEPGETGPPGRGLTGPTGAVGLPGPPGPSGLVGPQGSPGLPGQVGETGKPGAPGRDGASGKDGDRGSPGVPGSPGLPGPVGPKGEPGPTGAPGQAVVGLPGAKGEKGAPGGLAGDLVGEPGAKGDRGLPGPRGEKGEAGRAGEPGDPGEDGQKGAPGPKGFKGDPGVGVPGSPGPPGPPGVKGDLGLPGLPGAPGVVGFPGQTGPRGEMGQPGPSGERGLAGPPGREGIPGPLGPPGPPGSVGPPGASGLKGDKGDPGVGLPGPRGERGEPGIRGEDGRPGQEGPRGLTGPPGSRGERGEKGDVGSAGLKGDKGDSAVILGPPGPRGAKGDMGERGPRGLDGDKGPRGDNGDPGDKGSKGEPGDKGSAGLPGLRGLLGPQGQPGAAGIPGDPGSPGKDGVPGIRGEKGDVGFMGPRGLKGERGVKGACGLDGEKGDKGEAGPPGRPGLAGHKGEMGEPGVPGQSGAPGKEGLIGPKGDRGFDGQPGPKGDQGEKGERGTPGIGGFPGPSGNDGSAGPPGPPGSVGPRGPEGLQGQKGERGPPGERVVGAPGVPGAPGERGEQGRPGPAGPRGEKGEAALTEDDIRGFVRQEMSQHCACQGQFIASGSRPLPSYAADTAGSQLHAVPVLRVSHAEEEERVPPEDDEYSEYSEYSVEEYQDPEAPWDSDDPCSLPLDEGSCTAYTLRWYHRAVTGSTEACHPFVYGGCGGNANRFGTREACERRCPPRVVQSQGTGTAQD

SEQ ID NO: 3 - DNA, 20 bp, Homo sapiens
  source 1..20: mol_type = genomic DNA
accccacagtggggccacta

SEQ ID NO: 4 - DNA, 20 bp, Homo sapiens
  source 1..20: mol_type = genomic DNA
gtcaccaatcctgtccctag

SEQ ID NO: 5 - DNA, 20 bp, Homo sapiens
  source 1..20: mol_type = genomic DNA
ggggccactagggacaggat

SEQ ID NO: 6 - DNA, 1188 bp, synthetic construct
  misc_feature 1..1188: note = EF1a promoter
  source 1..1188: mol_type = other DNA
gtgaggctccggtgcccgtcagtgggcagagcgcacatcgcccacagtccccgagaagttggggggaggggtcggcaattgaaccggtgcctagagaaggtggcgcggggtaaactgggaaagtgatgtcgtgtactggctccgcctttttcccgagggtgggggagaaccgtatataagtgcagtagtcgccgtgaacgttctttttcgcaacgggtttgccgccagaacacaggtaagtgccgtgtgtggttcccgcgggcctggcctctttacgggttatggcccttgcgtgccttgaattacttccacgcccctggctgcagtacgtgattcttgatcccgagcttcgggttggaagtgggtgggagagttcgaggccttgcgcttaaggagccccttcgcctcgtgcttgagttgaggcctggcttgggcgctggggccgccgcgtgcgaatctggtggcaccttcgcgcctgtctcgctgctttcgataagtctctagccatttaaaatttttgatgacctgctgcgacgctttttttctggcaagatagtcttgtaaatgcgggccaagatctgcacactggtatttcggtttttggggccgcgggcggcgacggggcccgtgcgtcccagcgcacatgttcggcgaggcggggcctgcgagcgcggccaccgagaatcggacgggggtagtctcaagctggccggcctgctctggtgcctggcctcgcgccgccgtgtatcgccccgccctgggcggcaaggctggcccggtcggcaccagttgcgtgagcggaaagatggccgcttcccggccctgctgcagggagctcaaaatggaggacgcggcgctcgggagagcgggcgggtgagtcacccacacaaaggaaaagggcctttccgtcctcagccgtcgcttcatgtgactccacggagtaccgggcgccgtccaggcacctcgattagttctcgagcttttggagtacgtcgtctttaggttggggggaggggttttatgcgatggagtttccccacactgagtgggtggagactgaagttaggccagcttggcacttgatgtaattctccttggaatttgccctttttgagtttggatcttggttcattctcaagcctcagacagtggttcaaagtttttttcttccatttcaggtgtcgtgaa